European Patent Specification EP 3 458 080 B1, published July 10, 2024. Title: POLYPEPTIDES MODULATING SIGLEC DEPENDENT IMMUNE RESPONSES. Applicant: Octpharma AG. The sequence listing filed with the application follows.

SEQUENCE LISTING (21 sequences)

SEQ ID NO: 1 - protein, 2050 aa, Homo sapiens
SLSCRPPMVKLVCPADNLRAEGLECTKTCQNYDLECMSMGCVSGCLCPPGMVRHENRCVALERCPCFHQGKEYAPGETVKIGCNTCVCQDRKWNCTDHVCDATCSTIGMAHYLTFDGLKYLFPGECQYVLVQDYCGSNPGTFRILVGNKGCSHPSVKCKKRVTILVEGGEIELFDGEVNVKRPMKDETHFEVVESGRYIILLLGKALSVVWDRHLSISVVLKQTYQEKVCGLCGNFDGIQNNDLTSSNLQVEEDPVDFGNSWKVSSQCADTRKVPLDSSPATCHNNIMKQTMVDSSCRILTSDVFQDCNKLVDPEPYLDVCIYDTCSCESIGDCACFCDTIAAYAHVCAQHGKVVTWRTATLCPQSCEERNLRENGYECEWRYNSCAPACQVTCQHPEPLACPVQCVEGCHAHCPPGKILDELLQTCVDPEDCPVCEVAGRRFASGKKVTLNPSDPEHCQICHCDVVNLTCEACQEPGGLVVPPTDAPVSPTTLYVEDISEPPLHDFYCSRLLDLVFLLDGSSRLSEAEFEVLKAFVVDMMERLRISQKWVRVAVVEYHDGSHAYIGLKDRKRPSELRRIASQVKYAGSQVASTSEVLKYTLFQIFSKIDRPEASRITLLLMASQEPQRMSRNFVRYVQGLKKKKVIVIPVGIGPHANLKQIRLIEKQAPENKAFVLSSVDELEQQRDEIVSYLCDLAPEAPPPTLPPDMAQVTVGPGLLGVSTLGPKRNSMVLDVAFVLEGSDKIGEADFNRSKEFMEEVIQRMDVGQDSIHVTVLQYSYMVTVEYPFSEAQSKGDILQRVREIRYQGGNRTNTGLALRYLSDHSFLVSQGDREQAPNLVYMVTGNPASDEIKRLPGDIQVVPIGVGPNANVQELERIGWPNAPILIQDFETLPREAPDLVLQRCCSGEGLQIPTLSPAPDCSQPLDVILLLDGSSSFPASYFDEMKSFAKAFISKANIGPRLTQVSVLQYGSITTIDVPWNVVPEKAHLLSLVDVMQREGGPSQIGDALGFAVRYLTSEMHGARPGASKAVVILVTDVSVDSVDAAADAARSNRVTVFPIGIGDRYDAAQLRILAGPAGDSNVVKLQRIEDLPTMVTLGNSFLHKLCSGFVRICMDEDGNEKRPGDVWTLPDQCHTVTCQPDGQTLLKSHRVNCDRGLRPSCPNSQSPVKVEETCGCRWTCPCVCTGSSTRHIVTFDGQNFKLTGSCSYVLFQNKEQDLEVILHNGACSPGARQGCMKSIEVKHSALSVELHSDMEVTVNGRLVSVPYVGGNMEVNVYGAIMHEVRFNHLGHIFTFTPQNNEFQLQLSPKTFASKTYGLCGICDENGANDFMLRDGTVTTDWKTLVQEWTVQRPGQTCQPILEEQCLVPDSSHCQVLLLPLFAECHKVLAPATFYAICQQDSCHQEQVCEVIASYAHLCRTNGVCVDWRTPDFCAMSCPPSLVYNHCEHGCPRHCDGNVSSCGDHPSEGCFCPPDKVMLEGSCVPEEACTQCIGEDGVQHQFLEAWVPDHQPCQICTCLSGRKVNCTTQPCPTAKAPTCGLCEVARLRQNADQCCPEYECVCDPVSCDLPPVPHCERGLQPTLTNPGECRPNFTCACRKEECKRVSPPSCPPHRLPTLRKTQCCDEYECACNCVNSTVSCPLGYLASTATNDCGCTTTTCLPDKVCVHRSTIYPVGQFWEEGCDVCTCTDMEDAVMGLRVAQCSQKPCEDSCRSGFTYVLHEGECCGRCLPSACEVVTGSPRGDSQSSWKSVGSQWASPENPCLINECVRVKEEVFIQQRNVSCPQLEVPVCPSGFQLSCKTSACCPSCRCERMEACMLNGTVIGPGKTVMIDVCTTCRCMVQVGVISGFKLECRKTTCNPCPLGYKEENNTGECCGRCLPTACTIQLRGGQIMTLKRDETLQDGCDTHFCKVNERGEYFWEKRVTGCPPFDEHKCLAEGGKIMKIPGTCCDTCEEPECNDITARLQYVKVGSCKSEVEVDIHYCQGKCASKAMYSIDINDVQDQCSCCSPTRTEPMQVALHCTNGSVVYHEVLNAMECKCSPRKCSK

SEQ ID NO: 2 - protein, 566 aa, Homo sapiens
SLSCRPPMVKLVCPADNLRAEGLECTKTCQNYDLECMSMGCVSGCLCPPGMVRHENRCVALERCPCFHQGKEYAPGETVKIGCNTCVCQDRKWNCTDHVCDATCSTIGMAHYLTFDGLKYLFPGECQYVLVQDYCGSNPGTFRILVGNKGCSHPSVKCKKRVTILVEGGEIELFDGEVNVKRPMKDETHFEVVESGRYIILLLGKALSVVWDRHLSISVVLKQTYQEKVCGLCGNFDGIQNNDLTSSNLQVEEDPVDFGNSWKVSSQCADTRKVPLDSSPATCHNNIMKQTMVDSSCRILTSDVFQDCNKLVDPEPYLDVCIYDTCSCESIGDCACFCDTIAAYAHVCAQHGKVVTWRTATLCPQSCEERNLRENGYECEWRYNSCAPACQVTCQHPEPLACPVQCVEGCHAHCPPGKILDELLQTCVDPEDCPVCVAGRRFASGKKVTLNPSDPEHCQICHCDVVNLTCEACQEPGGLVVPPTDAPVSPTTLYVEDISEPPLHQEPGGLVVPPTDAPVSPTTLYVEDISEPPLHQEPGGLVVPPTDAPVSPTTLYVEDISEPPLH

SEQ ID NO: 3 - protein, 588 aa, Homo sapiens
MIPARFAGVLLALALILPGTLCSLSCRPPMVKLVCPADNLRAEGLECTKTCQNYDLECMSMGCVSGCLCPPGMVRHENRCVALERCPCFHQGKEYAPGETVKIGCNTCVCQDRKWNCTDHVCDATCSTIGMAHYLTFDGLKYLFPGECQYVLVQDYCGSNPGTFRILVGNKGCSHPSVKCKKRVTILVEGGEIELFDGEVNVKRPMKDETHFEVVESGRYIILLLGKALSVVWDRHLSISVVLKQTYQEKVCGLCGNFDGIQNNDLTSSNLQVEEDPVDFGNSWKVSSQCADTRKVPLDSSPATCHNNIMKQTMVDSSCRILTSDVFQDCNKLVDPEPYLDVCIYDTCSCESIGDCACFCDTIAAYAHVCAQHGKVVTWRTATLCPQSCEERNLRENGYECEWRYNSCAPACQVTCQHPEPLACPVQCVEGCHAHCPPGKILDELLQTCVDPEDCPVCVAGRRFASGKKVTLNPSDPEHCQICHCDVVNLTCEACQEPGGLVVPPTDAPVSPTTLYVEDISEPPLHQEPGGLVVPPTDAPVSPTTLYVEDISEPPLHQEPGGLVVPPTDAPVSPTTLYVEDISEPPLH

SEQ ID NO: 4 - protein, 1330 aa, Homo sapiens
MIPARFAGVLLALALILPGTLCAEGTRGRSSTARCSLFGSDFVNTFDGSMYSFAGYCSYLLAGGCQKRSFSIIGDFQNGKRVSLSVYLGEFFDIHLFVNGTVTQGDQRVSMPYASKGLYLETEAGYYKLSGEAYGFVARIDGSGNFQVLLSDRYFNKTCGLCGNFNIFAEDDFMTQEGTLTSDPYDFANSWALSSGEQWCERASPPSSSCNISSGEMQKGLWEQCQLLKSTSVFARCHPLVDPEPFVALCEKTLCECAGGLECACPALLEYARTCAQEGMVLYGWTDHSACSPVCPAGMEYRQCVSPCARTCQSLHINEMCQERCVDGCSCPEGQLLDEGLCVESTECPCVHSGKRYPPGTSLSRDCNTCICRNSQWICSNEECPGECLVTGQSHFKSFDNRYFTFSGICQYLLARDCQDHSFSIVIETVQCADDRDAVCTRSVTVRLPGLHNSLVKLKHGAGVAMDGQDVQLPLLKGDLRIQHTVTASVRLSYGEDLQMDWDGRGRLLVKLSPVYAGKTCGLCGNYNGNQGDDFLTPSGLAEPRVEDFGNAWKLHGDCQDLQKQHSDPCALNPRMTRFSEEACAVLTSPTFEACHRAVSPLPYLRNCRYDVCSCSDGRECLCGALASYAAACAGRGVRVAWREPGRCELNCPKGQVYLQCGTPCNLTCRSLSYPDEECNEACLEGCFCPPGLYMDERGDCVPKAQCPCYYDGEIFQPEDIFSDHHTMCYCEDGFMHCTMSGVPGSLLPDAVLSSPLSHRSKRSLSCRPPMVKLVCPADNLRAEGLECTKTCQNYDLECMSMGCVSGCLCPPGMVRHENRCVALERCPCFHQGKEYAPGETVKIGCNTCVCQDRKWNCTDHVCDATCSTIGMAHYLTFDGLKYLFPGECQYVLVQDYCGSNPGTFRILVGNKGCSHPSVKCKKRVTILVEGGEIELFDGEVNVKRPMKDETHFEVVESGRYIILLLGKALSVVWDRHLSISVVLKQTYQEKVCGLCGNFDGIQNNDLTSSNLQVEEDPVDFGNSWKVSSQCADTRKVPLDSSPATCHNNIMKQTMVDSSCRILTSDVFQDCNKLVDPEPYLDVCIYDTCSCESIGDCACFCDTIAAYAHVCAQHGKVVTWRTATLCPQSCEERNLRENGYECEWRYNSCAPACQVTCQHPEPLACPVQCVEGCHAHCPPGKILDELLQTCVDPEDCPVCEVAGRRFASGKKVTLNPSDPEHCQICHCDVVNLTCEACQEPGGLVVPPTDAPVSPTTLYVEDISEPPLHQEPGGLVVPPTDAPVSPTTLYVEDISEPPLHQEPGGLVVPPTDAPVSPTTLYVEDISEPPLH

SEQ ID NO: 5 - protein, 1423 aa, Homo sapiens
MIPARFAGVLLALALILPGTLCAEGTRGRSSTARCSLFGSDFVNTFDGSMYSFAGYCSYLLAGGCQKRSFSIIGDFQNGKRVSLSVYLGEFFDIHLFVNGTVTQGDQRVSMPYASKGLYLETEAGYYKLSGEAYGFVARIDGSGNFQVLLSDRYFNKTCGLCGNFNIFAEDDFMTQEGTLTSDPYDFANSWALSSGEQWCERASPPSSSCNISSGEMQKGLWEQCQLLKSTSVFARCHPLVDPEPFVALCEKTLCECAGGLECACPALLEYARTCAQEGMVLYGWTDHSACSPVCPAGMEYRQCVSPCARTCQSLHINEMCQERCVDGCSCPEGQLLDEGLCVESTECPCVHSGKRYPPGTSLSRDCNTCICRNSQWICSNEECPGECLVTGQSHFKSFDNRYFTFSGICQYLLARDCQDHSFSIVIETVQCADDRDAVCTRSVTVRLPGLHNSLVKLKHGAGVAMDGQDVQLPLLKGDLRIQHTVTASVRLSYGEDLQMDWDGRGRLLVKLSPVYAGKTCGLCGNYNGNQGDDFLTPSGLAEPRVEDFGNAWKLHGDCQDLQKQHSDPCALNPRMTRFSEEACAVLTSPTFEACHRAVSPLPYLRNCRYDVCSCSDGRECLCGALASYAAACAGRGVRVAWREPGRCELNCPKGQVYLQCGTPCNLTCRSLSYPDEECNEACLEGCFCPPGLYMDERGDCVPKAQCPCYYDGEIFQPEDIFSDHHTMCYCEDGFMHCTMSGVPGSLLPDAVLSSPLSHRSKRSLSCRPPMVKLVCPADNLRAEGLECTKTCQNYDLECMSMGCVSGCLCPPGMVRHENRCVALERCPCFHQGKEYAPGETVKIGCNTCVCQDRKWNCTDHVCDATCSTIGMAHYLTFDGLKYLFPGECQYVLVQDYCGSNPGTFRILVGNKGCSHPSVKCKKRVTILVEGGEIELFDGEVNVKRPMKDETHFEVVESGRYIILLLGKALSVVWDRHLSISVVLKQTYQEKVCGLCGNFDGIQNNDLTSSNLQVEEDPVDFGNSWKVSSQCADTRKVPLDSSPATCHNNIMKQTMVDSSCRILTSDVFQDCNKLVDPEPYLDVCIYDTCSCESIGDCACFCDTIAAYAHVCAQHGKVVTWRTATLCPQSCEERNLRENGYECEWRYNSCAPACQVTCQHPEPLACPVQCVEGCHAHCPPGKILDELLQTCVDPEDCPVCEVAGRRFASGKKVTLNPSDPEHCQICHCDVVNLTCEACQEPGGLVVPPTDAPVSPTTLYVEDISEPPLHQEPGGLVVPPTDAPVSPTTLYVEDISEPPLHQEPGGLVVPPTDAPVPTTLYVEDISEPPLHEEPECNDITARLQYVKVGSCKSEVEVDIHYCQGKCASKAMYSIDINDVQDQCSCCSPTRTEPMQVALHCTNGSVVYHEVLNAMECKCSPRKCSK

SEQ ID NO: 6 - protein, 62 aa, Homo sapiens
KVTLNPSDPEHCQICHCDVVNLTCEACQEPGGLVVPPTDAPVSPTTLYVEDISEPPLHGSAW

SEQ ID NO: 7 - protein, 124 aa, Homo sapiens
KVTLNPSDPEHCQICHCDVVNLTCEACQEPGGLVVPPTDAPVSPTTLYVEDISEPPLHQEPGGLVVPPTDAPVSPTTLYVEDISEPPLHQEPGGLVVPPTDAPVSPTTLYVEDISEPPLHGSAW

SEQ ID NO: 8 - protein, 23 aa, Homo sapiens
  misc_feature (6)..(6): Xaa can be any naturally occurring amino acid
  misc_feature (10)..(10): Xaa can be any naturally occurring amino acid
  misc_feature (14)..(14): Xaa can be any naturally occurring amino acid
  misc_feature (17)..(19): Xaa can be any naturally occurring amino acid
  misc_feature (21)..(21): Xaa can be any naturally occurring amino acid
VVPPTXAPVXPTTXYVXXXSXPP

SEQ ID NO: 9 - protein, 23 aa, Homo sapiens
VVPPTDAPVSPTTLYVEDISEPP

SEQ ID NO: 10 - protein, 26 aa, Homo sapiens
  misc_feature (5)..(5): Xaa can be any naturally occurring amino acid
  misc_feature (8)..(9): Xaa can be any naturally occurring amino acid
  misc_feature (11)..(11): Xaa can be any naturally occurring amino acid
  misc_feature (15)..(15): Xaa can be any naturally occurring amino acid
  misc_feature (17)..(20): Xaa can be any naturally occurring amino acid
  misc_feature (24)..(25): Xaa can be any naturally occurring amino acid
PPPTXPPXXAXVTVXPXXXXVSTXXP

SEQ ID NO: 11 - protein, 26 aa, Homo sapiens
PPPTLPPDMAQVTVGPGLLGVSTLGP

SEQ ID NO: 12 - protein, 47 aa, Homo sapiens
  misc_feature (6)..(9): Xaa can be any naturally occurring amino acid
  misc_feature (12)..(12): Xaa can be any naturally occurring amino acid
  misc_feature (15)..(17): Xaa can be any naturally occurring amino acid
  misc_feature (20)..(20): Xaa can be any naturally occurring amino acid
  misc_feature (22)..(23): Xaa can be any naturally occurring amino acid
  misc_feature (27)..(28): Xaa can be any naturally occurring amino acid
  misc_feature (32)..(32): Xaa can be any naturally occurring amino acid
  misc_feature (35)..(37): Xaa can be any naturally occurring amino acid
  misc_feature (39)..(41): Xaa can be any naturally occurring amino acid
  misc_feature (44)..(47): Xaa can be any naturally occurring amino acid
VSSTSXXXXSTXPSXXXAAXTXXTSSXXPPSXPVXXXSXXXTTXXXX

SEQ ID NO: 13 - protein, 47 aa, Homo sapiens
VSSTSNNLISTIPSDNLAAGTDDTSSLGPPSMPVHYDSQLDTTLFGK

SEQ ID NO: 14 - protein, 20 aa, Homo sapiens
  misc_feature (1)..(3): Xaa can be any naturally occurring amino acid
  misc_feature (7)..(7): Xaa can be any naturally occurring amino acid
  misc_feature (9)..(14): Xaa can be any naturally occurring amino acid
  misc_feature (16)..(16): Xaa can be any naturally occurring amino acid
  misc_feature (18)..(20): Xaa can be any naturally occurring amino acid
XXXATTXPXXXXXXTXPXXX

SEQ ID NO: 15 - protein, 20 aa, Homo sapiens
QFNATTIPENDIEKTDPWFA

SEQ ID NO: 16 - protein, 10 aa, Homo sapiens
  misc_feature (1)..(2): Xaa can be any naturally occurring amino acid
  misc_feature (8)..(10): Xaa can be any naturally occurring amino acid
XXTTAATXXX

SEQ ID NO: 17 - protein, 10 aa, Homo sapiens
LGTTAATELK

SEQ ID NO: 18 - protein, 17 aa, Homo sapiens
  misc_feature (1)..(2): Xaa can be any naturally occurring amino acid
  misc_feature (6)..(8): Xaa can be any naturally occurring amino acid
  misc_feature (10)..(10): Xaa can be any naturally occurring amino acid
  misc_feature (12)..(14): Xaa can be any naturally occurring amino acid
  misc_feature (17)..(17): Xaa can be any naturally occurring amino acid
XXPTPXXXSXSXXXEAX

SEQ ID NO: 19 - protein, 17 aa, Homo sapiens
QSPTPHGLSLSDLQEAK

SEQ ID NO: 20 - protein, 37 aa, Homo sapiens
  misc_feature (2)..(10): Xaa can be any naturally occurring amino acid
  misc_feature (12)..(12): Xaa can be any naturally occurring amino acid
  misc_feature (15)..(16): Xaa can be any naturally occurring amino acid
  misc_feature (19)..(23): Xaa can be any naturally occurring amino acid
  misc_feature (25)..(26): Xaa can be any naturally occurring amino acid
  misc_feature (28)..(31): Xaa can be any naturally occurring amino acid
  misc_feature (33)..(34): Xaa can be any naturally occurring amino acid
  misc_feature (36)..(37): Xaa can be any naturally occurring amino acid
VXXXXXXXXXTXTSXXSPXXXXXVXXSXXXXTXXAXX

SEQ ID NO: 21 - protein, 37 aa, Homo sapiens
VHIYQKDLFFTETSDGSPGHLDLVEGSLLQGTEGAIK